European Patent Application EP 4 163 293 A1, published April 12, 2023. Title: NOVEL NUCLEOSIDE TRIPHOSPHATE TRANSPORTER AND USES THEREOF. Applicant: THE SCRIPPS RESEARCH INSTITUTE. The sequence listing filed with the application follows.

SEQUENCE LISTING (264 sequences)

SEQ ID NO: 1 - protein, 575 aa, Phaeodactylum tricornutum
MRPYPTIALISVFLSAATRISATSSHQASALPVKKGTHVPDSPKLSKLYIMAKTKSVSSSFDPPRGGSTVAPTTPLATGGALRKVRQAVFPIYGNQEVTKFLLIGSIKFFIILALTLTRDTKDTLIVTQCGAEAIAFLKIYGVLPAATAFIALYSKMSNAMGKKMLFYSTCIPFFTFFGLFDVFIYPNAERLHPSLEAVQAILPGGAASGGMAVLAKIATHWTSALFYVMAEIYSSVSVGLLFWQFANDVVNVDQAKRFYPLFAQMSGLAPVLAGQYVVRFASKAVNFEASMHRLTAAVTFAGIMICIFYQLSSSYVERTESAKPAADNEQSIKPKKKKPKMSMVESGKFLASSQYLRLIAMLVLGYGLSINFTEIMWKSLVKKQYPDPLDYQRFMGNFSSAVGLSTCIVIFFGVHVIRLLGWKVGALATPGIMAILALPFFACILLGLDSPARLEIAVIFGTIQSLLSKTSKYALFDPTTQMAYIPLDDESKVKGKAAIDVLGSRIGKSGGSLIQQGLVFVFGNIINAAPVVGVVYYSVLVAWMSAAGRLSGLFQAQTEMDKADKMEAKTNKEK

SEQ ID NO: 2 - DNA, 1536 bp, Artificial Sequence
  Description of Artificial Sequence: Synthetic polynucleotide
atgggtggtagcaccgttgcaccgaccacaccgctggcaaccggtggtgcactgcgtaaagttcgtcaggcagtttttccgatttatggcaatcaagaagtgaccaaatttctgctgattggcagcatcaaattctttattatcctggcactgaccctgacccgtgataccaaagataccctgattgttacccagtgtggtgcagaagcaattgcatttctgaaaatctatggtgttctgcctgcagcaaccgcatttattgcactgtatagcaaaatgagcaacgcaatgggcaaaaaaatgctgttttatagcacctgtatcccgttctttaccttttttggtctgttcgatgtgttcatttatccgaatgccgaacgtctgcatccgagcctggaagcagttcaggcaattctgcctggtggtgccgcaagcggtggtatggcagttctggcaaaaattgcaacccattggaccagcgcactgttttatgttatggcagaaatctatagcagcgttagcgttggtctgctgttttggcagtttgcaaatgatgttgttaatgtggatcaggccaaacgtttttatccgctgtttgcacagatgagcggtctggcaccggttctggcaggtcagtatgttgttcgttttgcaagcaaagccgttaattttgaagcaagcatgcatcgtctgaccgcagcagttacctttgcaggtattatgatctgcatcttttatcagctgagcagctcatatgttgaacgtaccgaaagcgcaaaaccggcagcagataatgaacagagcattaaaccgaagaaaaaaaaaccgaaaatgtcgatggtggaaagcggtaaatttctggcaagcagccagtatctgcgtctgattgcaatgctggttctgggttatggtctgagcattaactttaccgaaatcatgtggaaaagcctggtgaaaaaacagtatccggatccgctggattatcagcgttttatgggtaattttagcagcgcagttggtctgagtacctgcattgttatcttttttggcgtgcatgttattcgtctgctgggttggaaagttggtgccctggcaacaccgggtattatggccattctggcactgccgttttttgcatgtattctgctgggcctggatagtccggcacgtctggaaattgcagttatttttggcaccattcagagcctgctgagcaaaaccagcaaatatgcactgtttgatccgaccacccagatggcatatatcccgctggatgatgaaagcaaagttaaaggcaaagcagccattgatgttctgggtagccgtattggtaaatcaggtggtagcctgattcagcagggtctggtttttgtttttggcaatattatcaatgccgcaccggttgttggtgttgtgtattatagcgttctggttgcatggatgagtgcagcaggtcgtctgagtggtctgtttcaggcacagaccgaaatggataaagcagataaaatggaagccaaaaccaacaaagaaaaatga

SEQ ID NO: 3 - DNA, 1536 bp, Phaeodactylum tricornutum
atgggaggcagtactgttgcaccaactacaccgttggcaaccggcggtgcgctccgcaaagtgcgacaagccgtctttcccatctacggaaaccaagaagtcaccaaatttctgctcatcggatccattaaattctttataatcttggcactcacgctcacgcgtgataccaaggacacgttgattgtcacgcaatgtggtgccgaagcgattgcctttctcaaaatatacggggtgctacccgcagcgaccgcatttatcgcgctctattccaaaatgtccaacgccatgggcaaaaaaatgctattttattccacttgcattcctttctttacctttttcgggctgtttgatgttttcatttacccgaacgcggagcgactgcaccctagtttggaagccgtgcaggcaattctcccgggcggtgccgcatctggcggcatggcggttctggccaagattgcgacacactggacatcggccttattttacgtcatggcggaaatatattcttccgtatcggtggggctattgttttggcagtttgcgaacgacgtcgtcaacgtggatcaggccaagcgcttttatccattatttgctcaaatgagtggcctcgctccagttttagcgggccagtatgtggtacggtttgccagcaaagcggtcaactttgaggcatccatgcatcgactcacggcggccgtaacatttgctggtattatgatttgcatcttttaccaactcagttcgtcatatgtggagcgaacggaatcagcaaagccagcggcagataacgagcagtctatcaaaccgaaaaagaagaaacccaaaatgtccatggttgaatcggggaaatttctcgcgtcaagtcagtacctgcgtctaattgccatgctggtgctgggatacggcctcagtattaactttaccgaaatcatgtggaaaagcttggtgaagaaacaatatccagacccgctagattatcaacgatttatgggtaacttctcgtcagcggttggtttgagcacatgcattgttattttcttcggtgtgcacgtgatccgtttgttggggtggaaagtcggagcgttggctacacctgggatcatggccattctagcgttacccttttttgcttgcattttgttgggtttggatagtccagcacgattggagatcgccgtaatctttggaacaattcagagtttgctgagcaaaacctccaagtatgcccttttcgaccctaccacacaaatggcttatattcctctggacgacgaatcaaaggtcaaaggaaaagcggcaattgatgttttgggatcgcggattggcaagagtggaggctcactgatccagcagggcttggtctttgtttttggaaatatcattaatgccgcacctgtagtaggggttgtctactacagtgtccttgttgcgtggatgagcgcagctggccgactaagtgggctttttcaagcacaaacagaaatggataaggccgacaaaatggaggcaaagaccaacaaagaaaagtag

SEQ ID NO: 4 - protein, 511 aa, Phaeodactylum tricornutum
MGGSTVAPTTPLATGGALRKVRQAVFPIYGNQEVTKFLLIGSIKFFIILALTLTRDTKDTLIVTQCGAEAIAFLKIYGVLPAATAFIALYSKMSNAMGKKMLFYSTCIPFFTFFGLFDVFIYPNAERLHPSLEAVQAILPGGAASGGMAVLAKIATHWTSALFYVMAEIYSSVSVGLLFWQFANDVVNVDQAKRFYPLFAQMSGLAPVLAGQYVVRFASKAVNFEASMHRLTAAVTFAGIMICIFYQLSSSYVERTESAKPAADNEQSIKPKKKKPKMSMVESGKFLASSQYLRLIAMLVLGYGLSINFTEIMWKSLVKKQYPDPLDYQRFMGNFSSAVGLSTCIVIFFGVHVIRLLGWKVGALATPGIMAILALPFFACILLGLDSPARLEIAVIFGTIQSLLSKTSKYALFDPTTQMAYIPLDDESKVKGKAAIDVLGSRIGKSGGSLIQQGLVFVFGNIINAAPVVGVVYYSVLVAWMSAAGRLSGLFQAQTEMDKADKMEAKTNKEK

SEQ ID NO: 5 - DNA, 1599 bp, Artificial Sequence
  Description of Artificial Sequence: Synthetic polynucleotide
atgagaccatttccgacgattgccttgatttcggtttttctttcggcggcgactcgcatttcggcaggaggcagtactgttgcaccaactacaccgttggcaaccggcggtgcgctccgcaaagtgcgacaagccgtctttcccatctacggaaaccaagaagtcaccaaatttctgctcatcggatccattaaattctttataatcttggcactcacgctcacgcgtgataccaaggacacgttgattgtcacgcaatgtggtgccgaagcgattgcctttctcaaaatatacggggtgctacccgcagcgaccgcatttatcgcgctctattccaaaatgtccaacgccatgggcaaaaaaatgctattttattccacttgcattcctttctttacctttttcgggctgtttgatgttttcatttacccgaacgcggagcgactgcaccctagtttggaagccgtgcaggcaattctcccgggcggtgccgcatctggcggcatggcggttctggccaagattgcgacacactggacatcggccttattttacgtcatggcggaaatatattcttccgtatcggtggggctattgttttggcagtttgcgaacgacgtcgtcaacgtggatcaggccaagcgcttttatccattatttgctcaaatgagtggcctcgctccagttttagcgggccagtatgtggtacggtttgccagcaaagcggtcaactttgaggcatccatgcatcgactcacggcggccgtaacatttgctggtattatgatttgcatcttttaccaactcagttcgtcatatgtggagcgaacggaatcagcaaagccagcggcagataacgagcagtctatcaaaccgaaaaagaagaaacccaaaatgtccatggttgaatcggggaaatttctcgcgtcaagtcagtacctgcgtctaattgccatgctggtgctgggatacggcctcagtattaactttaccgaaatcatgtggaaaagcttggtgaagaaacaatatccagacccgctagattatcaacgatttatgggtaacttctcgtcagcggttggtttgagcacatgcattgttattttcttcggtgtgcacgtgatccgtttgttggggtggaaagtcggagcgttggctacacctgggatcatggccattctagcgttacccttttttgcttgcattttgttgggtttggatagtccagcacgattggagatcgccgtaatctttggaacaattcagagtttgctgagcaaaacctccaagtatgcccttttcgaccctaccacacaaatggcttatattcctctggacgacgaatcaaaggtcaaaggaaaagcggcaattgatgttttgggatcgcggattggcaagagtggaggctcactgatccagcagggcttggtctttgtttttggaaatatcattaatgccgcacctgtagtaggggttgtctactacagtgtccttgttgcgtggatgagcgcagctggccgactaagtgggctttttcaagcacaaacagaaatggataaggccgacaaaatggaggcaaagaccaacaaagaaaagtag

SEQ ID NO: 6 - protein, 532 aa, Artificial Sequence
  Description of Artificial Sequence: Synthetic polypeptide
MRPFPTIALISVFLSAATRISAGGSTVAPTTPLATGGALRKVRQAVFPIYGNQEVTKFLLIGSIKFFIILALTLTRDTKDTLIVTQCGAEAIAFLKIYGVLPAATAFIALYSKMSNAMGKKMLFYSTCIPFFTFFGLFDVFIYPNAERLHPSLEAVQAILPGGAASGGMAVLAKIATHWTSALFYVMAEIYSSVSVGLLFWQFANDVVNVDQAKRFYPLFAQMSGLAPVLAGQYVVRFASKAVNFEASMHRLTAAVTFAGIMICIFYQLSSSYVERTESAKPAADNEQSIKPKKKKPKMSMVESGKFLASSQYLRLIAMLVLGYGLSINFTEIMWKSLVKKQYPDPLDYQRFMGNFSSAVGLSTCIVIFFGVHVIRLLGWKVGALATPGIMAILALPFFACILLGLDSPARLEIAVIFGTIQSLLSKTSKYALFDPTTQMAYIPLDDESKVKGKAAIDVLGSRIGKSGGSLIQQGLVFVFGNIINAAPVVGVVYYSVLVAWMSAAGRLSGLFQAQTEMDKADKMEAKTNKEK

SEQ ID NO: 7 - DNA, 1665 bp, Artificial Sequence
  Description of Artificial Sequence: Synthetic polynucleotide
atgacttcctctcatcaagcaagtgcacttcctctcaaaaagggaacgcatgtcccggactctccgaagttgtcaaagctatatatcatggccaaaaccaagagtgtatcctcgtccttcgacccccctcggggaggcagtactgttgcaccaactacaccgttggcaaccggcggtgcgctccgcaaagtgcgacaagccgtctttcccatctacggaaaccaagaagtcaccaaatttctgctcatcggatccattaaattctttataatcttggcactcacgctcacgcgtgataccaaggacacgttgattgtcacgcaatgtggtgccgaagcgattgcctttctcaaaatatacggggtgctacccgcagcgaccgcatttatcgcgctctattccaaaatgtccaacgccatgggcaaaaaaatgctattttattccacttgcattcctttctttacctttttcgggctgtttgatgttttcatttacccgaacgcggagcgactgcaccctagtttggaagccgtgcaggcaattctcccgggcggtgccgcatctggcggcatggcggttctggccaagattgcgacacactggacatcggccttattttacgtcatggcggaaatatattcttccgtatcggtggggctattgttttggcagtttgcgaacgacgtcgtcaacgtggatcaggccaagcgcttttatccattatttgctcaaatgagtggcctcgctccagttttagcgggccagtatgtggtacggtttgccagcaaagcggtcaactttgaggcatccatgcatcgactcacggcggccgtaacatttgctggtattatgatttgcatcttttaccaactcagttcgtcatatgtggagcgaacggaatcagcaaagccagcggcagataacgagcagtctatcaaaccgaaaaagaagaaacccaaaatgtccatggttgaatcggggaaatttctcgcgtcaagtcagtacctgcgtctaattgccatgctggtgctgggatacggcctcagtattaactttaccgaaatcatgtggaaaagcttggtgaagaaacaatatccagacccgctagattatcaacgatttatgggtaacttctcgtcagcggttggtttgagcacatgcattgttattttcttcggtgtgcacgtgatccgtttgttggggtggaaagtcggagcgttggctacacctgggatcatggccattctagcgttacccttttttgcttgcattttgttgggtttggatagtccagcacgattggagatcgccgtaatctttggaacaattcagagtttgctgagcaaaacctccaagtatgcccttttcgaccctaccacacaaatggcttatattcctctggacgacgaatcaaaggtcaaaggaaaagcggcaattgatgttttgggatcgcggattggcaagagtggaggctcactgatccagcagggcttggtctttgtttttggaaatatcattaatgccgcacctgtagtaggggttgtctactacagtgtccttgttgcgtggatgagcgcagctggccgactaagtgggctttttcaagcacaaacagaaatggataaggccgacaaaatggaggcaaagaccaacaaagaaaagtag

SEQ ID NO: 8 - protein, 554 aa, Artificial Sequence
  Description of Artificial Sequence: Synthetic polypeptide
MTSSHQASALPLKKGTHVPDSPKLSKLYIMAKTKSVSSSFDPPRGGSTVAPTTPLATGGALRKVRQAVFPIYGNQEVTKFLLIGSIKFFIILALTLTRDTKDTLIVTQCGAEAIAFLKIYGVLPAATAFIALYSKMSNAMGKKMLFYSTCIPFFTFFGLFDVFIYPNAERLHPSLEAVQAILPGGAASGGMAVLAKIATHWTSALFYVMAEIYSSVSVGLLFWQFANDVVNVDQAKRFYPLFAQMSGLAPVLAGQYVVRFASKAVNFEASMHRLTAAVTFAGIMICIFYQLSSSYVERTESAKPAADNEQSIKPKKKKPKMSMVESGKFLASSQYLRLIAMLVLGYGLSINFTEIMWKSLVKKQYPDPLDYQRFMGNFSSAVGLSTCIVIFFGVHVIRLLGWKVGALATPGIMAILALPFFACILLGLDSPARLEIAVIFGTIQSLLSKTSKYALFDPTTQMAYIPLDDESKVKGKAAIDVLGSRIGKSGGSLIQQGLVFVFGNIINAAPVVGVVYYSVLVAWMSAAGRLSGLFQAQTEMDKADKMEAKTNKEK

SEQ ID NO: 9 - DNA, 3013 bp, Artificial Sequence
  Description of Artificial Sequence: Synthetic polynucleotide
  modified_base (2349)..(2349): Any unnatural nucleotide
aacgccagcaacgcggcctttttacggttcctggccttttgctggccttttgctcacatgttctttcctgcgttatcccctgattctgtggataaccgtattaccgcctttgagtgagctgataccgctcgccgcagccgaacgaccgagcgcagcgagtcagtgagcgaggaagcggaagagcgcctgatgcggtattttctccttacgcatctgtgcggtatttcacaccgcatatggtgcactctcagtacaatctgctctgatgccgcatagttaagccagtatacactccgctatcgctacgtgactgggtcatggctgcgccccgacacccgccaacacccgctgacgcgccctgacgggcttgtctgctcccggcatccgcttacagacaagctgtgaccgtctccgggagctgcatgtgtcagaggttttcaccgtcatcaccgaaacgcgcgaggcagctgcggtaaagctcatcagcgtggtcgtgaagcgattcacagatgtctgcctgttcatccgcgtccagctcgttgagtttctccagaagcgttaatgtctggcttctgataaagcgggccatgttaagggcggttttttcctgtttggtcactgatgcctccgtgtaagggggatttctgttcatgggggtaatgataccgatgaaacgagagaggatgctcacgatacgggttactgatgatgaacatgcccggttactggaacgttgtgagggtaaacaactggcggtatggatgcggcgggaccagagaaaaatcactcagggtcaatgccagcgcttcgttaatacagatgtaggtgttccacagggtagccagcagcatcctgcgatgcagatccggaacataatggtgcagggcgctgacttccgcgtttccagactttacgaaacacggaaaccgaagaccattcatgttgttgctcaggtcgcagacgttttgcagcagcagtcgcttcacgttcgctcgcgtatcggtgattcattctgctaaccagtaaggcaaccccgccagcctagccgggtcctcaacgacaggagcacgatcatgcgcacccgtggccaggacccaacgctgcccgaaattcttgaagacgaaagggcctcgtgatacgcctatttttataggttaatgtcatgataataatggtttcttagacgtcaggtggcacttttcggggaaatgtgcgcggaacccctatttgtttatttttctaaatacattcaaatatgtatccgctcatgagacaataaccctgataaatgcttcaataatattgaaaaaggaagagtatgagtattcaacatttccgtgtcgcccttattcccttttttgcggcattttgccttcctgtttttgctcacccagaaacgctggtgaaagtaaaagatgctgaagatcagttgggtgcacgagtgggttacatcgaactggatctcaacagcggtaagatccttgagagttttcgccccgaagaacgttttccaatgatgagcacttttaaagttctgctatgtggcgcggtattatcccgtgttgacgccgggcaagagcaactcggtcgccgcatacactattctcagaatgacttggttgagtactcaccagtcacagaaaagcatcttacggatggcatgacagtaagagaattatgcagtgctgccataaccatgagtgataacactgcggccaacttacttctgacaacgatcggaggaccgaaggagctaaccgcttttttgcacaacatgggggatcatgtaactcgccttgatcgttgggaaccggagctgaatgaagccataccaaacgacgagcgtgacaccacgatgcctgcagcaatggcaacaacgttgcgcaaactattaactggcgaactacttactctagcttcccggcaacaattaatagactggatggaggcggataaagttgcaggaccacttctgcgctcggcccttccggctggctggtttattgctgataaatctggagccggtgagcgtggctctcgcggtatcattgcagcactggggccagatggtaagccctcccgtatcgtagttatctacacgacggggagtcaggcaactatggatgaacgaaatagacagatcgctgagataggtgcctcactgattaagcattggtaactgtcagaccaagtttactcatatatactttagattgatttaaaacttcatttttaatttaaaaggatctaggtgaagatcctttttgataatctcatgaccaaaatcccttaacgtgagttttcgttggctttacactttatgcttccggctcgtatgttgtgtggaantgtgagcggataacaatttcacacaggaaacagccactgagcgtcagaccccgtagaaaagatcaaaggatcttcttgagatcctttttttctgcgcgtaatctgctgcttgcaaacaaaaaaaccaccgctaccagcggtggtttgtttgccggatcaagagctaccaactctttttccgaaggtaactggcttcagcagagcgcagataccaaatactgtccttctagtgtagccgtagttaggccaccacttcaagaactctgtagcaccgcctacatacctcgctctgctaatcctgttaccagtggctgctgccagtggcgataagtcgtgtcttaccgggttggactcaagacgatagttaccggataaggcgcagcggtcgggctgaacggggggttcgtgcacacagcccagcttggagcgaacgacctacaccgaactgagatacctacagcgtgagctatgagaaagcgccacgcttcccgaagggagaaaggcggacaggtatccggtaagcggcagggtcggaacaggagagcgcacgagggagcttccagggggaaacgcctggtatctttatagtcctgtcgggtttcgccacctctgacttgagcgtcgatttttgtgatgctcgtcaggggggcggagcctatggaaa

SEQ ID NO: 10 - DNA, 20 bp, Artificial Sequence
  Description of Artificial Sequence: Synthetic primer
gggaggcagtactgttgcac

SEQ ID NO: 11 - DNA, 45 bp, Artificial Sequence
  Description of Artificial Sequence: Synthetic primer
ggtatatctccttattaaagttaaacaaaattatttctacagggg

SEQ ID NO: 12 - DNA, 20 bp, Artificial Sequence
  Description of Artificial Sequence: Synthetic primer
taatacgactcactataggg

SEQ ID NO: 13 - DNA, 19 bp, Artificial Sequence
  Description of Artificial Sequence: Synthetic primer
gctagttattgctcagcgg

SEQ ID NO: 14 - DNA, 22 bp, Artificial Sequence
  Description of Artificial Sequence: Synthetic primer
ttacattaattgcgttgcgctc

SEQ ID NO: 15 - DNA, 31 bp, Artificial Sequence
  Description of Artificial Sequence: Synthetic primer
ttttggcggatggcatttgagaagcacacgg

SEQ ID NO: 16 - DNA, 25 bp, Artificial Sequence
  Description of Artificial Sequence: Synthetic primer
attctcaccaataaaaaacgcccgg

SEQ ID NO: 17 - DNA, 36 bp, Artificial Sequence
  Description of Artificial Sequence: Synthetic primer
cctgtagaaataattttgtttaactttaataaggag

SEQ ID NO: 18 - DNA, 20 bp, Artificial Sequence
  Description of Artificial Sequence: Synthetic primer
ccccgcgcgttggccgattc

SEQ ID NO: 19 - DNA, 19 bp, Artificial Sequence
  Description of Artificial Sequence: Synthetic primer
gaagggcaatcagctgttg

SEQ ID NO: 20 - DNA, 21 bp, Artificial Sequence
  Description of Artificial Sequence: Synthetic primer
cagggcagggtcgttaaatag

SEQ ID NO: 21 - DNA, 52 bp, Artificial Sequence
  Description of Artificial Sequence: Synthetic primer
gacaccatcgaatggcgcaaaacctttcgcggtatggcatgatagcgcccgg

SEQ ID NO: 22 - DNA, 52 bp, Artificial Sequence
  Description of Artificial Sequence: Synthetic primer
ccgggcgctatcatgccataccgcgaaaggttttgcgccattcgatggtgtc

SEQ ID NO: 23 - DNA, 51 bp, Artificial Sequence
  Description of Artificial Sequence: Synthetic primer
atttttctaaatacattcaaatatgtatccgctcatgagacaataaccctg

SEQ ID NO: 24 - DNA, 51 bp, Artificial Sequence
  Description of Artificial Sequence: Synthetic primer
cagggttattgtctcatgagcggatacatatttgaatgtatttagaaaaat

SEQ ID NO: 25 - DNA, 52 bp, Artificial Sequence
  Description of Artificial Sequence: Synthetic primer
ttaggcaccccaggctttacactttatgcttccggctggtatgttgtgtgga

SEQ ID NO: 26 - DNA, 52 bp, Artificial Sequence
  Description of Artificial Sequence: Synthetic primer
tccacacaacataccagccggaagcataaagtgtaaagcctggggtgcctaa

SEQ ID NO: 27 - DNA, 52 bp, Artificial Sequence
  Description of Artificial Sequence: Synthetic primer
ctaggcaccccaggctttacactttatgcttccggctggtataatgtgtgga

SEQ ID NO: 28 - DNA, 52 bp, Artificial Sequence
  Description of Artificial Sequence: Synthetic primer
tccacacattataccagccggaagcataaagtgtaaagcctggggtgcctag

SEQ ID NO: 29 - DNA, 24 bp, Artificial Sequence
  Description of Artificial Sequence: Synthetic primer
ggggataacgcaggaaagaacatg

SEQ ID NO: 30 - DNA, 22 bp, Artificial Sequence
  Description of Artificial Sequence: Synthetic primer
gcacttttcggggaaatgtgcg

SEQ ID NO: 31 - DNA, 75 bp, Artificial Sequence
  Description of Artificial Sequence: Synthetic primer
aattgcggcctatatggatgttggaaccgtaagagaaatagacaggcggtcctgtgacggaagatcacttcgcag

SEQ ID NO: 32 - DNA, 46 bp, Artificial Sequence
  Description of Artificial Sequence: Synthetic primer
tgctcacatgttctttcctgcgttatccccgcgtggtgaaccaggc

SEQ ID NO: 33 - DNA, 28 bp, Artificial Sequence
  Description of Artificial Sequence: Synthetic primer
accgcctgtctatttctcttacggttcc

SEQ ID NO: 34 - DNA, 49 bp, Artificial Sequence
  Description of Artificial Sequence: Synthetic primer
cgcgcttaatgcgccgctacagggcgcgtcgattggtgccagcgcgcag

SEQ ID NO: 35 - DNA, 43 bp, Artificial Sequence
  Description of Artificial Sequence: Synthetic primer
ggtatatctccttattaaagttaaacaaaattatttctacagg

SEQ ID NO: 36 - DNA, 21 bp, Artificial Sequence
  Description of Artificial Sequence: Synthetic primer
cagccacgtttctgcgaaaac

SEQ ID NO: 37 - DNA, 20 bp, Artificial Sequence
  Description of Artificial Sequence: Synthetic primer
tacagcggttccttactggc

SEQ ID NO: 38 - DNA, 26 bp, Artificial Sequence
  Description of Artificial Sequence: Synthetic primer
gggtggtgaatgtgaaaccagtaacg

SEQ ID NO: 39 - DNA, 21 bp, Artificial Sequence
  Description of Artificial Sequence: Synthetic primer
ctgggtgtttacttcggtctg

SEQ ID NO: 40 - DNA, 21 bp, Artificial Sequence
  Description of Artificial Sequence: Synthetic primer
ggccgtaatatccagctgaac

SEQ ID NO: 41 - DNA, 20 bp, Artificial Sequence
  Description of Artificial Sequence: Synthetic primer
actagggtgcagtcgctccg

SEQ ID NO: 42 - DNA, 22 bp, Artificial Sequence
  Description of Artificial Sequence: Synthetic primer
ttaacctaggctgctgccaccg

SEQ ID NO: 43 - DNA, 57 bp, Artificial Sequence
  Description of Artificial Sequence: Synthetic primer
gcgcaacgcaattaatgtaattctgaaatgagctgttgacaattaatcatcggctcg

SEQ ID NO: 44 - DNA, 56 bp, Artificial Sequence
  Description of Artificial Sequence: Synthetic primer
aacaaaattatttctacaggtccacacattatacgagccgatgattaattgtcaac

SEQ ID NO: 45 - DNA, 58 bp, Artificial Sequence
  Description of Artificial Sequence: Synthetic primer
gcgcaacgcaattaatgtaatcataaaaaatttatttgctttcaggaaaatttttctg

SEQ ID NO: 46 - DNA, 59 bp, Artificial Sequence
  Description of Artificial Sequence: Synthetic primer
aacaaaattatttctacaggtgaatctattatacagaaaaattttcctgaaagcaaata

SEQ ID NO: 47 - DNA, 56 bp, Artificial Sequence
  Description of Artificial Sequence: Synthetic primer
gcgcaacgcaattaatgtaattatctctggcggtgttgacataaataccactggcg

SEQ ID NO: 48 - DNA, 57 bp, Artificial Sequence
  Description of Artificial Sequence: Synthetic primer
aacaaaattatttctacaggtgtgctcagtatcaccgccagtggtatttatgtcaac

SEQ ID NO: 49 - DNA, 58 bp, Artificial Sequence
  Description of Artificial Sequence: Synthetic primer
gcgcaacgcaattaatgtaattttaaaaaattcatttgctaaacgcttcaaattctcg

SEQ ID NO: 50 - DNA, 55 bp, Artificial Sequence
  Description of Artificial Sequence: Synthetic primer
aacaaaattatttctacaggtgaagtatattatacgagaatttgaagcgtttagc

SEQ ID NO: 51 - DNA, 21 bp, Artificial Sequence
  Description of Artificial Sequence: Synthetic primer
tggggtgcctaatgagtgagc

SEQ ID NO: 52 - DNA, 26 bp, Artificial Sequence
  Description of Artificial Sequence: Synthetic primer
ctatgaccatgattacgccaagcttg

SEQ ID NO: 53 - DNA, 24 bp, Artificial Sequence
  Description of Artificial Sequence: Synthetic primer
tctcgcggtatcattgcagcactg

SEQ ID NO: 54 - DNA, 18 bp, Artificial Sequence
  Description of Artificial Sequence: Synthetic primer
gccacgctcaccggctcc

SEQ ID NO: 55 - DNA, 21 bp, Artificial Sequence
  Description of Artificial Sequence: Synthetic primer
aacgaaaactcacgttaaggg

SEQ ID NO: 56 - DNA, 17 bp, Artificial Sequence
  Description of Artificial Sequence: Synthetic primer
ccactgagcgtcagacc

SEQ ID NO: 57 - DNA, 30 bp, Artificial Sequence
  Description of Artificial Sequence: Synthetic primer
gagacccgtcgttgacaattaatcatcggc

SEQ ID NO: 58 - DNA, 31 bp, Artificial Sequence
  Description of Artificial Sequence: Synthetic primer
gagaccattctcaccaataaaaaacgcccgg

SEQ ID NO: 59 - DNA, 30 bp, Artificial Sequence
  Description of Artificial Sequence: Synthetic primer
cggggtaccatggacaagaagtactccatt

SEQ ID NO: 60 - DNA, 34 bp, Artificial Sequence
  Description of Artificial Sequence: Synthetic primer
ctagtctagattacaccttcctcttcttcttggg

SEQ ID NO: 61 - DNA, 33 bp, Artificial Sequence
  Description of Artificial Sequence: Synthetic primer
ctccggggaaaccgccgaagccacgcggctcaa

SEQ ID NO: 62 - DNA, 44 bp, Artificial Sequence
  Description of Artificial Sequence: Synthetic primer
cttcggcggtttccccggagtcgaacaggagggcgccaatgagg

SEQ ID NO: 63 - DNA, 40 bp, Artificial Sequence
  Description of Artificial Sequence: Synthetic primer
aggaagaagacgtctcacgcatcttactgcgcagatacgc

SEQ ID NO: 64 - DNA, 60 bp, Artificial Sequence
  Description of Artificial Sequence: Synthetic primer
aagatgcgtgagacgtcttcttcctcgtctcggtcgacagttcataggtgattgctcagg

SEQ ID NO: 65 - DNA, 26 bp, Artificial Sequence
  Description of Artificial Sequence: Synthetic primer
gtcccaaatcgcagccaatcacattg

SEQ ID NO: 66 - DNA, 28 bp, Artificial Sequence
  Description of Artificial Sequence: Synthetic primer
gtcctgaccatcgtattggttatctggc

SEQ ID NO: 67 - DNA, 26 bp, Artificial Sequence
  Description of Artificial Sequence: Synthetic primer
atttagagggcagtgccagctcgtta

SEQ ID NO: 68 - DNA, 26 bp, Artificial Sequence
  Description of Artificial Sequence: Synthetic primer
ctgcattcaggtaggcatcatgcgca

SEQ ID NO: 69 - DNA, 26 bp, Artificial Sequence
  Description of Artificial Sequence: Synthetic primer
ctgggctacctgcaagattagcgatg

SEQ ID NO: 70 - DNA, 25 bp, Artificial Sequence
  Description of Artificial Sequence: Synthetic primer
tgaaggactgggcagaggccccctt

SEQ ID NO: 71 - DNA, 26 bp, Artificial Sequence
  Description of Artificial Sequence: Synthetic primer
cgtaggtgtctttgctcagttgaagc

SEQ ID NO: 72 - DNA, 27 bp, Artificial Sequence
  Description of Artificial Sequence: Synthetic primer
tagccatctcattactaaagatctcct

SEQ ID NO: 73 - DNA, 43 bp, Artificial Sequence
  Description of Artificial Sequence: Synthetic primer
cgatatcgttggtctcaacgacacaattgtaaaggttagatct

SEQ ID NO: 74 - DNA, 43 bp, Artificial Sequence
  Description of Artificial Sequence: Synthetic primer
caacgatatcggtctcacactgactgggcctttcgttttatct

SEQ ID NO: 75 - DNA, 23 bp, Artificial Sequence
  Description of Artificial Sequence: Synthetic primer
gcaatcacctatgaactgtcgac

SEQ ID NO: 76 - DNA, 69 bp, Artificial Sequence
  Description of Artificial Sequence: Synthetic primer
aggaggaaggacgtctcatgcgccccgcattcacacaatgtagtgatcagttttagagctagaaatagc

SEQ ID NO: 77 - DNA, 69 bp, Artificial Sequence
  Description of Artificial Sequence: Synthetic primer
aggaggaaggacgtctcatgcgccccgcattccaggatgggtaccacccgttttagagctagaaatagc

SEQ ID NO: 78 - DNA, 69 bp, Artificial Sequence
  Description of Artificial Sequence: Synthetic primer
aggaggaaggacgtctcatgcgccccgcattcacacaatgtagtcatcagttttagagctagaaatagc

SEQ ID NO: 79 - DNA, 69 bp, Artificial Sequence
  Description of Artificial Sequence: Synthetic primer
aggaggaaggacgtctcatgcgccccgcattccaggatgggcaccagccgttttagagctagaaatagc

SEQ ID NO: 80 - DNA, 69 bp, Artificial Sequence
  Description of Artificial Sequence: Synthetic primer
aggaggaaggacgtctcatgcgccccgcattccatgatgggcaccacccgttttagagctagaaatagc

SEQ ID NO: 81 - DNA, 69 bp, Artificial Sequence
  Description of Artificial Sequence: Synthetic primer
aggaggaaggacgtctcatgcgccccgcattcacacaatgtatagatcagttttagagctagaaatagc

SEQ ID NO: 82 - DNA, 69 bp, Artificial Sequence
  Description of Artificial Sequence: Synthetic primer
aggaggaaggacgtctcatgcgccccgcattccaggatgggcaccatccgttttagagctagaaatagc

SEQ ID NO: 83 - DNA, 69 bp, Artificial Sequence
  Description of Artificial Sequence: Synthetic primer
aggaggaaggacgtctcatgcgccccgcattgttgtgtggaaatgtgaggttttagagctagaaatagc

SEQ ID NO: 84 - DNA, 69 bp, Artificial Sequence
  Description of Artificial Sequence: Synthetic primer
aggaggaaggacgtctcatgcgccccgcatttgtcactactctgaccaggttttagagctagaaatagc

SEQ ID NO: 85 - DNA, 69 bp, Artificial Sequence
  Description of Artificial Sequence: Synthetic primer
aggaggaaggacgtctcatgcgccccgcatttgtcactactctgaccaagttttagagctagaaatagc

SEQ ID NO: 86 - DNA, 69 bp, Artificial Sequence
  Description of Artificial Sequence: Synthetic primer
aggaggaaggacgtctcatgcgccccgcattcacacaatgtactcatcagttttagagctagaaatagc

SEQ ID NO: 87 - DNA, 69 bp, Artificial Sequence
  Description of Artificial Sequence: Synthetic primer
aggaggaaggacgtctcatgcgccccgcattccaagatgggcaccacccgttttagagctagaaatagc

SEQ ID NO: 88 - DNA, 69 bp, Artificial Sequence
  Description of Artificial Sequence: Synthetic primer
aggaggaaggacgtctcatgcgccccgcattcacacaatgtattgatcagttttagagctagaaatagc

SEQ ID NO: 89 - DNA, 69 bp, Artificial Sequence
  Description of Artificial Sequence: Synthetic primer
aggaggaaggacgtctcatgcgccccgcattcacacaatgtataaatcagttttagagctagaaatagc

SEQ ID NO: 90 - DNA, 69 bp, Artificial Sequence
  Description of Artificial Sequence: Synthetic primer
aggaggaaggacgtctcatgcgccccgcattccaggatggggaccacccgttttagagctagaaatagc

SEQ ID NO: 91 - DNA, 69 bp, Artificial Sequence
  Description of Artificial Sequence: Synthetic primer
aggaggaaggacgtctcatgcgccccgcattttcacaatactttctttagttttagagctagaaatagc

SEQ ID NO: 92 - DNA, 43 bp, Artificial Sequence
  Description of Artificial Sequence: Synthetic primer
gcatttcacacaatgtaggatcagttttagagctagaaatagc

SEQ ID NO: 93 - DNA, 38 bp, Artificial Sequence
  Description of Artificial Sequence: Synthetic primer
tgatcctacattgtgtgaaatgcggggcgcatcttact

SEQ ID NO: 94 - DNA, 43 bp, Artificial Sequence
  Description of Artificial Sequence: Synthetic primer
gcattaccaggatgggaccacccgttttagagctagaaatagc

SEQ ID NO: 95 - DNA, 38 bp, Artificial Sequence
  Description of Artificial Sequence: Synthetic primer
gggtggtcccatcctggtaatgcggggcgcatcttact

SEQ ID NO: 96 - DNA, 43 bp, Artificial Sequence
  Description of Artificial Sequence: Synthetic primer
gcatttcacacaatgtagcatcagttttagagctagaaatagc

SEQ ID NO: 97 - DNA, 38 bp, Artificial Sequence
  Description of Artificial Sequence: Synthetic primer
tgatgctacattgtgtgaaatgcggggcgcatcttact

SEQ ID NO: 98 - DNA, 43 bp, Artificial Sequence
  Description of Artificial Sequence: Synthetic primer
gcattaccaggatgggcaccaccgttttagagctagaaatagc

SEQ ID NO: 99 - DNA, 38 bp, Artificial Sequence
  Description of Artificial Sequence: Synthetic primer
ggtggtgcccatcctggtaatgcggggcgcatcttact

SEQ ID NO: 100 - DNA, 43 bp, Artificial Sequence
  Description of Artificial Sequence: Synthetic primer
gcattaccagatgggcaccacccgttttagagctagaaatagc

SEQ ID NO: 101 - DNA, 38 bp, Artificial Sequence
  Description of Artificial Sequence: Synthetic primer
gggtggtgcccatctggtaatgcggggcgcatcttact

SEQ ID NO: 102 - DNA, 43 bp, Artificial Sequence
  Description of Artificial Sequence: Synthetic primer
gcatttcacacaatgtaagatcagttttagagctagaaatagc

SEQ ID NO: 103 - DNA, 38 bp, Artificial Sequence
  Description of Artificial Sequence: Synthetic primer
tgatcttacattgtgtgaaatgcggggcgcatcttact

SEQ ID NO: 104 - DNA, 43 bp, Artificial Sequence
  Description of Artificial Sequence: Synthetic primer
gcatttgttgtgtggaatgtgaggttttagagctagaaatagc

SEQ ID NO: 105 - DNA, 38 bp, Artificial Sequence
  Description of Artificial Sequence: Synthetic primer
ctcacattccacacaacaaatgcggggcgcatcttact

SEQ ID NO: 106 - DNA, 43 bp, Artificial Sequence
  Description of Artificial Sequence: Synthetic primer
gcattttgtcactactctgaccggttttagagctagaaatagc

SEQ ID NO: 107 - DNA, 38 bp, Artificial Sequence
  Description of Artificial Sequence: Synthetic primer
cggtcagagtagtgacaaaatgcggggcgcatcttact

SEQ ID NO: 108 - DNA, 43 bp, Artificial Sequence
  Description of Artificial Sequence: Synthetic primer
gcattttgtcactactctgaccagttttagagctagaaatagc

SEQ ID NO: 109 - DNA, 38 bp, Artificial Sequence
  Description of Artificial Sequence: Synthetic primer
tggtcagagtagtgacaaaatgcggggcgcatcttact

SEQ ID NO: 110 - DNA, 43 bp, Artificial Sequence
  Description of Artificial Sequence: Synthetic primer
gcatttcacacaatgtaccatcagttttagagctagaaatagc

SEQ ID NO: 111 - DNA, 38 bp, Artificial Sequence
  Description of Artificial Sequence: Synthetic primer
tgatggtacattgtgtgaaatgcggggcgcatcttact

SEQ ID NO: 112 - DNA, 43 bp, Artificial Sequence
  Description of Artificial Sequence: Synthetic primer
gcatttcacacaatgtatgatcagttttagagctagaaatagc

SEQ ID NO: 113 - DNA, 38 bp, Artificial Sequence
  Description of Artificial Sequence: Synthetic primer
tgatcatacattgtgtgaaatgcggggcgcatcttact

SEQ ID NO: 114 - DNA, 43 bp, Artificial Sequence
  Description of Artificial Sequence: Synthetic primer
gcatttcacacaatgtataatcagttttagagctagaaatagc

SEQ ID NO: 115 - DNA, 38 bp, Artificial Sequence
  Description of Artificial Sequence: Synthetic primer
tgattatacattgtgtgaaatgcggggcgcatcttact

SEQ ID NO: 116 - DNA, 43 bp, Artificial Sequence
  Description of Artificial Sequence: Synthetic primer
gcattattcacaatacttctttagttttagagctagaaatagc

SEQ ID NO: 117 - DNA, 38 bp, Artificial Sequence
  Description of Artificial Sequence: Synthetic primer
taaagaagtattgtgaataatgcggggcgcatcttact

SEQ ID NO: 118 - DNA, 47 bp, Artificial Sequence
  Description of Artificial Sequence: Synthetic primer
agaaggaagacgtctcactgtcgaccaaaaaagcctgctcgttgagc

SEQ ID NO: 119 - DNA, 40 bp, Artificial Sequence
  Description of Artificial Sequence: Synthetic primer
aagaaggacgtctcaacagtagtggcagcggctaactaag

SEQ ID NO: 120 - DNA, 44 bp, Artificial Sequence
  Description of Artificial Sequence: Synthetic primer
aggagaggacgtctctcgaccaaaaaagcctgctcgttgagcag

SEQ ID NO: 121 - DNA, 59 bp, Artificial Sequence
  Description of Artificial Sequence: Synthetic primer
agtaagatgcgccccgcattgaccaggatgggcaccacccgttttagagctagaaatag

SEQ ID NO: 122 - DNA, 59 bp, Artificial Sequence
  Description of Artificial Sequence: Synthetic primer
ctatttctagctctaaaacgggtggtgcccatcctggtcaatgcggggcgcatcttact

SEQ ID NO: 123 - DNA, 39 bp, Artificial Sequence
  Description of Artificial Sequence: Synthetic primer
gttttagagctagaaatagcaagttaaaataaggctagt

SEQ ID NO: 124 - DNA, 20 bp, Artificial Sequence
  Description of Artificial Sequence: Synthetic primer
aatgcggggcgcatcttact

SEQ ID NO: 125 - DNA, 22 bp, Artificial Sequence
  Description of Artificial Sequence: Synthetic primer
cattggcaccggtctactaaac

SEQ ID NO: 126 - DNA, 22 bp, Artificial Sequence
  Description of Artificial Sequence: Synthetic primer
aaacgtttagtagaccggtgcc

SEQ ID NO: 127 - DNA, 29 bp, Artificial Sequence
  Description of Artificial Sequence: Synthetic primer
cgcattcacacaatgtaagtatcagtttt

SEQ ID NO: 128 - DNA, 29 bp, Artificial Sequence
  Description of Artificial Sequence: Synthetic primer
ctctaaaactgatacttacattgtgtgaa

SEQ ID NO: 129 - DNA, 60 bp, Artificial Sequence
  Description of Artificial Sequence: Synthetic primer
gtttacgtcgccgtccagctcgaccaggatgggcaccaacccggtgaacagctcctcgcc

SEQ ID NO: 130 - DNA, 60 bp, Artificial Sequence
  Description of Artificial Sequence: Synthetic primer
gtttacgtcgccgtccagctcgaccaggatgggcaccagcccggtgaacagctcctcgcc

SEQ ID NO: 131 - DNA, 60 bp, Artificial Sequence
  Description of Artificial Sequence: Synthetic primer
gtttacgtcgccgtccagctcgaccaggatgggcaccatcccggtgaacagctcctcgcc

SEQ ID NO: 132 - DNA, 60 bp, Artificial Sequence
  Description of Artificial Sequence: Synthetic primer
gtttacgtcgccgtccagctcgaccaggatgggcaccaccccggtgaacagctcctcgcc

SEQ ID NO: 133 - DNA, 60 bp, Artificial Sequence
  Description of Artificial Sequence: Synthetic primer
gcatcgccctcgccctcgccggacacgctgaacttgtggccgtttacgtcgccgtccagc

SEQ ID NO: 134 - DNA, 60 bp, Artificial Sequence
  Description of Artificial Sequence: Synthetic primer
tgcagtttcatttgatgctcgatgagttatggtgagcaagggcgaggagctgttcaccgg

SEQ ID NO: 135 - DNA, 79 bp, Artificial Sequence
  Description of Artificial Sequence: Synthetic primer
ttaatacgactcactatagggaccaggatgggcaccaaccgttttagagctagaaatagcaagttaaaataaggctagt

SEQ ID NO: 136 - DNA, 79 bp, Artificial Sequence
  Description of Artificial Sequence: Synthetic primer
ttaatacgactcactatagggaccaggatgggcaccagccgttttagagctagaaatagcaagttaaaataaggctagt

SEQ ID NO: 137 - DNA, 79 bp, Artificial Sequence
  Description of Artificial Sequence: Synthetic primer
ttaatacgactcactatagggaccaggatgggcaccatccgttttagagctagaaatagcaagttaaaataaggctagt

SEQ ID NO: 138 - DNA, 62 bp, Artificial Sequence
  Description of Artificial Sequence: Synthetic primer
ttaatacgactcactatagggaccaggatgggcaccacccgttttagagctatgctgttttg

SEQ ID NO: 139 - DNA, 82 bp, Artificial Sequence
  Description of Artificial Sequence: Synthetic primer
aaaagcaccgactcggtgccactttttcaagttgataacggactagccttattttaacttgctatttctagctctaaaacgg

SEQ ID NO: 140 - DNA, 35 bp, Artificial Sequence
  Description of Artificial Sequence: Synthetic primer
aagaggaagaggttaatacgactcactatagggac

SEQ ID NO: 141 - DNA, 20 bp, Artificial Sequence
  Description of Artificial Sequence: Synthetic primer
aaaagcaccgactcggtgcc

SEQ ID NO: 142 - DNA, 41 bp, Artificial Sequence
  Description of Artificial Sequence: Synthetic primer
actagccttattttaacttgctatttctagctctaaaacgg

SEQ ID NO: 143 - DNA, 48 bp, Artificial Sequence
  Description of Artificial Sequence: Synthetic primer
aagaaggagaaggtctctagtggagcaagggcgaggagctgttcaccg

SEQ ID NO: 144 - DNA, 43 bp, Artificial Sequence
  Description of Artificial Sequence: Synthetic primer
aagagaagagaggtctcatcgtgtttacgtcgccgtccagctc

SEQ ID NO: 145 - DNA, 34 bp, Artificial Sequence
  Description of Artificial Sequence: Synthetic primer
atgggtctccagtggggccaacacttgtcactac

SEQ ID NO: 146 - DNA, 34 bp, Artificial Sequence
  Description of Artificial Sequence: Synthetic primer
atgggtctcttcgtttccggataacgggaaaagc

SEQ ID NO: 147 - DNA, 39 bp, Artificial Sequence
  Description of Artificial Sequence: Synthetic primer
atgggtctccagtggctcgagtacaactttaactcacac

SEQ ID NO: 148 - DNA, 39 bp, Artificial Sequence
  Description of Artificial Sequence: Synthetic primer
atgggtctcttcgttgattccattcttttgtttgtctgc

SEQ ID NO: 149 - DNA, 41 bp, Artificial Sequence
  Description of Artificial Sequence: Synthetic primer
atgggtctctcatagctgtttcctgtgtgaaattgttatcc

SEQ ID NO: 150 - DNA, 37 bp, Artificial Sequence
  Description of Artificial Sequence: Synthetic primer
atgggtctcaccccaggctttacactttatgcttccg

SEQ ID NO: 151 - DNA, 41 bp, Artificial Sequence
  Description of Artificial Sequence: Synthetic primer
atgggtctccagtggctgtttcctgtgtgaaattgttatcc

SEQ ID NO: 152 - DNA, 37 bp, Artificial Sequence
  Description of Artificial Sequence: Synthetic primer
atgggtctcttcgttggctttacactttatgcttccg

SEQ ID NO: 153 - DNA, 36 bp, Artificial Sequence
  Description of Artificial Sequence: Synthetic primer
atgggtctccagtggcacacaggaaacagctatgac

SEQ ID NO: 154 - DNA, 41 bp, Artificial Sequence
  Description of Artificial Sequence: Synthetic primer
atgggtctcttcgttgggttaagcttaactttaagaaggag

SEQ ID NO: 155 - DNA, 40 bp, Artificial Sequence
  Description of Artificial Sequence: Synthetic primer
atgggtctcacacaaactcgagtacaactttaactcacac

SEQ ID NO: 156 - DNA, 33 bp, Artificial Sequence
  Description of Artificial Sequence: Synthetic primer
atgggtctcgattccattcttttgtttgtctgc

SEQ ID NO: 157 - DNA, 29 bp, Artificial Sequence
  Description of Artificial Sequence: Synthetic primer
attggtctcggccgagcggttgaaggcac

SEQ ID NO: 158 - DNA, 29 bp, Artificial Sequence
  Description of Artificial Sequence: Synthetic primer
attggtctctctggaaccctttcgggtcg

SEQ ID NO: 159 - DNA, 19 bp, Artificial Sequence
  Description of Artificial Sequence: Synthetic primer
ggcgaggagctgttcaccg

SEQ ID NO: 160 - DNA, 21 bp, Artificial Sequence
  Description of Artificial Sequence: Synthetic primer
gtttacgtcgccgtccagctc

SEQ ID NO: 161 - DNA, 20 bp, Artificial Sequence
  Description of Artificial Sequence: Synthetic primer
ggccaacacttgtcactact

SEQ ID NO: 162 - DNA, 19 bp, Artificial Sequence
  Description of Artificial Sequence: Synthetic primer
tccggataacgggaaaagc

SEQ ID NO: 163 - DNA, 24 bp, Artificial Sequence
  Description of Artificial Sequence: Synthetic primer
ctcgagtacaactttaactcacac

SEQ ID NO: 164 - DNA, 24 bp, Artificial Sequence
  Description of Artificial Sequence: Synthetic primer
gattccattcttttgtttgtctgc

SEQ ID NO: 165 - DNA, 26 bp, Artificial Sequence
  Description of Artificial Sequence: Synthetic primer
ctgtttcctgtgtgaaattgttatcc

SEQ ID NO: 166 - DNA, 22 bp, Artificial Sequence
  Description of Artificial Sequence: Synthetic primer
ggctttacactttatgcttccg

SEQ ID NO: 167 - DNA, 26 bp, Artificial Sequence
  Description of Artificial Sequence: Synthetic primer
cccgggttattacatgcgctagcact

SEQ ID NO: 168 - DNA, 48 bp, Artificial Sequence
  Description of Artificial Sequence: Synthetic primer
gaaattaatacgactcactatagggttaagcttaactttaagaaggag

SEQ ID NO: 169 - DNA, 21 bp, Artificial Sequence
  Description of Artificial Sequence: Synthetic primer
tgcaagcagcagattacgcgc

SEQ ID NO: 170 - DNA, 24 bp, Artificial Sequence
  Description of Artificial Sequence: Synthetic primer
gtaactgtcagaccaagtttactc

SEQ ID NO: 171 - DNA, 60 bp, Artificial Sequence
  Description of Artificial Sequence: Synthetic oligonucleotide
  modified_base (22)..(22): dNaM
ggcgaggagctgttcaccgggntggtgcccatcctggtcgagctggacggcgacgtaaac

SEQ ID NO: 172 - DNA, 60 bp, Artificial Sequence
  Description of Artificial Sequence: Synthetic oligonucleotide
  modified_base (34)..(34): dNaM
gtttacgtcgccgtccagctcgaccaggatgggnaccaccccggtgaacagctcctcgcc

SEQ ID NO: 173 - DNA, 60 bp, Artificial Sequence
  Description of Artificial Sequence: Synthetic oligonucleotide
  modified_base (27)..(27): dNaM
gtttacgtcgccgtccagctcgaccangatgggcaccaccccggtgaacagctcctcgcc

SEQ ID NO: 174 - DNA, 60 bp, Artificial Sequence
  Description of Artificial Sequence: Synthetic oligonucleotide
  modified_base (39)..(39): dNaM
gtttacgtcgccgtccagctcgaccaggatgggcaccancccggtgaacagctcctcgcc

SEQ ID NO: 175 - DNA, 75 bp, Artificial Sequence
  Description of Artificial Sequence: Synthetic oligonucleotide
  modified_base (34)..(34): dNaM
ctgtttcctgtgtgaaattgttatccgctcacanttccacacaacatacgagccggaagcataaagtgtaaagcc

SEQ ID NO: 176 - DNA, 63 bp, Artificial Sequence
  Description of Artificial Sequence: Synthetic oligonucleotide
  modified_base (31)..(31): dNaM
ctcgagtacaactttaactcacacaatgtanagatcacggcagacaaacaaaagaatggaatc

SEQ ID NO: 177 - DNA, 58 bp, Artificial Sequence
  Description of Artificial Sequence: Synthetic oligonucleotide
  modified_base (31)..(31): dNaM
ccggataacgggaaaagcattgaacaccgcnggtcagagtagtgacaagtgttggcca

SEQ ID NO: 178 - DNA, 58 bp, Artificial Sequence
  Description of Artificial Sequence: Synthetic oligonucleotide
  modified_base (27)..(27): dNaM
ggccaacacttgtcactactctgaccnagggtgttcaatgcttttcccgttatccgga

SEQ ID NO: 179 - DNA, 60 bp, Artificial Sequence
  Description of Artificial Sequence: Synthetic oligonucleotide
  modified_base (34)..(34): dNaM
ggcgaggagctgttcaccggggtggtgcccatcntggtcgagctggacggcgacgtaaac

SEQ ID NO: 180 - DNA, 60 bp, Artificial Sequence
  Description of Artificial Sequence: Synthetic oligonucleotide
  modified_base (27)..(27): dNaM
ggcgaggagctgttcaccggggtggtncccatcctggtcgagctggacggcgacgtaaac

SEQ ID NO: 181 - DNA, 64 bp, Artificial Sequence
  Description of Artificial Sequence: Synthetic oligonucleotide
  modified_base (32)..(32): dNaM
gattccattcttttgtttgtctgccgtgattnatacattgtgtgagttaaagttgtactcgagt

SEQ ID NO: 182 - DNA, 134 bp, Artificial Sequence
  Description of Artificial Sequence: Synthetic polynucleotide
  modified_base (63)..(63): dNaM
cacacaggaaacagctatgacccgggttattacatgcgctagcacttggaattcacaatactntctttaaggaaaccatagtaaatctccttcttaaagttaagcttaaccctatagtgagtcgtattaatttc

SEQ ID NO: 183 - DNA, 63 bp, Artificial Sequence
  Description of Artificial Sequence: Synthetic oligonucleotide
  modified_base (32)..(32): dNaM
ctcgagtacaactttaactcacacaatgtaanaatcacggcagacaaacaaaagaatggaatc

SEQ ID NO: 184 - DNA, 63 bp, Artificial Sequence
  Description of Artificial Sequence: Synthetic oligonucleotide
  modified_base (32)..(32): dNaM
ctcgagtacaactttaactcacacaatgtaancatcacggcagacaaacaaaagaatggaatc

SEQ ID NO: 185 - DNA, 63 bp, Artificial Sequence
  Description of Artificial Sequence: Synthetic oligonucleotide
  modified_base (32)..(32): dNaM
ctcgagtacaactttaactcacacaatgtaangatcacggcagacaaacaaaagaatggaatc

SEQ ID NO: 186 - DNA, 63 bp, Artificial Sequence
  Description of Artificial Sequence: Synthetic oligonucleotide
  modified_base (32)..(32): dNaM
ctcgagtacaactttaactcacacaatgtcantgtcacggcagacaaacaaaagaatggaatc

SEQ ID NO: 187 - DNA, 63 bp, Artificial Sequence
  Description of Artificial Sequence: Synthetic oligonucleotide
  modified_base (32)..(32): dNaM
ctcgagtacaactttaactcacacaatgtacnaatcacggcagacaaacaaaagaatggaatc

SEQ ID NO: 188 - DNA, 63 bp, Artificial Sequence
  Description of Artificial Sequence: Synthetic oligonucleotide
  modified_base (32)..(32): dNaM
ctcgagtacaactttaactcacacaatgtacncatcacggcagacaaacaaaagaatggaatc

SEQ ID NO: 189 - DNA, 63 bp, Artificial Sequence
  Description of Artificial Sequence: Synthetic oligonucleotide
  modified_base (32)..(32): dNaM
ctcgagtacaactttaactcacacaatgtacngatcacggcagacaaacaaaagaatggaatc

SEQ ID NO: 190 - DNA, 63 bp, Artificial Sequence
  Description of Artificial Sequence: Synthetic oligonucleotide
  modified_base (32)..(32): dNaM
ctcgagtacaactttaactcacacaatgtacntatcacggcagacaaacaaaagaatggaatc

SEQ ID NO: 191 - DNA, 63 bp, Artificial Sequence
  Description of Artificial Sequence: Synthetic oligonucleotide
  modified_base (32)..(32): dNaM
ctcgagtacaactttaactcacacaatgtagnaatcacggcagacaaacaaaagaatggaatc

SEQ ID NO: 192 - DNA, 63 bp, Artificial Sequence
  Description of Artificial Sequence: Synthetic oligonucleotide
  modified_base (32)..(32): dNaM
ctcgagtacaactttaactcacacaatgtagncatcacggcagacaaacaaaagaatggaatc

SEQ ID NO: 193 - DNA, 63 bp, Artificial Sequence
  Description of Artificial Sequence: Synthetic oligonucleotide
  modified_base (32)..(32): dNaM
ctcgagtacaactttaactcacacaatgtagngatcacggcagacaaacaaaagaatggaatc

SEQ ID NO: 194 - DNA, 63 bp, Artificial Sequence
  Description of Artificial Sequence: Synthetic oligonucleotide
  modified_base (32)..(32): dNaM
ctcgagtacaactttaactcacacaatgtagntatcacggcagacaaacaaaagaatggaatc

SEQ ID NO: 195 - DNA, 63 bp, Artificial Sequence
  Description of Artificial Sequence: Synthetic oligonucleotide
  modified_base (32)..(32): dNaM
ctcgagtacaactttaactcacacaatgtatnaatcacggcagacaaacaaaagaatggaatc

SEQ ID NO: 196 - DNA, 63 bp, Artificial Sequence
  Description of Artificial Sequence: Synthetic oligonucleotide
  modified_base (32)..(32): dNaM
ctcgagtacaactttaactcacacaatgtatncatcacggcagacaaacaaaagaatggaatc

SEQ ID NO: 197 - DNA, 63 bp, Artificial Sequence
  Description of Artificial Sequence: Synthetic oligonucleotide
  modified_base (32)..(32): dNaM
ctcgagtacaactttaactcacacaatgtatngatcacggcagacaaacaaaagaatggaatc

SEQ ID NO: 198 - DNA, 63 bp, Artificial Sequence
  Description of Artificial Sequence: Synthetic oligonucleotide
  modified_base (32)..(32): dNaM
ctcgagtacaactttaactcacacaatgtatntatcacggcagacaaacaaaagaatggaatc

SEQ ID NO: 199 - DNA, 63 bp, Artificial Sequence
  Description of Artificial Sequence: Synthetic oligonucleotide
  modified_base (33)..(33): dNaM
ctcgagtacaactttaactcacacaatgtaagnatcacggcagacaaacaaaagaatggaatc

SEQ ID NO: 200 - DNA, 56 bp, Artificial Sequence
  Description of Artificial Sequence: Synthetic oligonucleotide
  modified_base (31)..(31): dNaM
ctctggaaccctttcgggtcgccggtttagnagaccggtgccttcaaccgctcggc

SEQ ID NO: 201 - DNA, 23 bp, Artificial Sequence
  Description of Artificial Sequence: Synthetic oligonucleotide
  modified_base (18)..(18): dC, dT, dA, dG, dTPT3 or dNaM
  See specification as filed for detailed description of substitutions and preferred embodiments
ctggtcctacccgtggtnggtcc

SEQ ID NO: 202 - DNA, 20 bp, Artificial Sequence
  Description of Artificial Sequence: Synthetic oligonucleotide
  Description of Combined DNA/RNA Molecule: Synthetic oligonucleotide
  modified_base (18)..(18): g, a, u or c
  See specification as filed for detailed description of substitutions and preferred embodiments
gaccaggatgggcaccancc

SEQ ID NO: 203 - RNA, 20 nt, Artificial Sequence
  Description of Artificial Sequence: Synthetic oligonucleotide
gaccaggaugggcaccaccc

SEQ ID NO: 204 - RNA, 18 nt, Artificial Sequence
  Description of Artificial Sequence: Synthetic oligonucleotide
guuguguggaaaugugag

SEQ ID NO: 205 - RNA, 18 nt, Artificial Sequence
  Description of Artificial Sequence: Synthetic oligonucleotide
uguuguguggaaugugag

SEQ ID NO: 206 - DNA, 22 bp, Artificial Sequence
  Description of Artificial Sequence: Synthetic oligonucleotide
  Description of Combined DNA/RNA Molecule: Synthetic oligonucleotide
  modified_base (16)..(16): dTPT3
guatgttgtgtggaantgtgag

SEQ ID NO: 207 - DNA, 13 bp, Artificial Sequence
  Description of Artificial Sequence: Synthetic oligonucleotide
  CDS (1)..(12)
tcacatttccaca

SEQ ID NO: 208 - protein, 4 aa, Artificial Sequence
  Description of Artificial Sequence: Synthetic peptide
SHFH

SEQ ID NO: 209 - DNA, 22 bp, Artificial Sequence
  Description of Artificial Sequence: Synthetic oligonucleotide
  modified_base (14)..(14): dNaM
tcacacaatgtagngatcacgg

SEQ ID NO: 210 - DNA, 22 bp, Artificial Sequence
  Description of Artificial Sequence: Synthetic oligonucleotide
  modified_base (12)..(12): dNaM
accaggatgggnaccaccccgg

SEQ ID NO: 211 - DNA, 22 bp, Artificial Sequence
  Description of Artificial Sequence: Synthetic oligonucleotide
  modified_base (14)..(14): dNaM
tcacacaatgtagncatcacgg

SEQ ID NO: 212 - DNA, 22 bp, Artificial Sequence
  Description of Artificial Sequence: Synthetic oligonucleotide
  modified_base (17)..(17): dTPT3
accaggatgggcaccancccgg

SEQ ID NO: 213 - DNA, 22 bp, Artificial Sequence
  Description of Artificial Sequence: Synthetic oligonucleotide
  modified_base (5)..(5): dNaM
accangatgggcaccaccccgg

SEQ ID NO: 214 - DNA, 22 bp, Artificial Sequence
  Description of Artificial Sequence: Synthetic oligonucleotide
  modified_base (13)..(13): dNaM
tcacacaatgtanagatcacgg

SEQ ID NO: 215 - DNA, 22 bp, Artificial Sequence
  Description of Artificial Sequence: Synthetic oligonucleotide
  modified_base (17)..(17): dNaM
accaggatgggcaccancccgg

SEQ ID NO: 216 - DNA, 22 bp, Artificial Sequence
  Description of Artificial Sequence: Synthetic oligonucleotide
  modified_base (13)..(13): dTPT3
tgttgtgtggaantgtgagcgg

SEQ ID NO: 217 - DNA, 22 bp, Artificial Sequence
  Description of Artificial Sequence: Synthetic oligonucleotide
  modified_base (18)..(18): dTPT3
ttgtcactactctgaccngcgg

SEQ ID NO: 218 - DNA, 22 bp, Artificial Sequence
  Description of Artificial Sequence: Synthetic oligonucleotide
  modified_base (18)..(18): dNaM
ttgtcactactctgaccnaggg

SEQ ID NO: 219 - DNA, 22 bp, Artificial Sequence
  Description of Artificial Sequence: Synthetic oligonucleotide
  modified_base (14)..(14): dNaM
tcacacaatgtacncatcacgg

SEQ ID NO: 220 - DNA, 22 bp, Artificial Sequence
  Description of Artificial Sequence: Synthetic oligonucleotide
  modified_base (5)..(5): dTPT3
accangatgggcaccaccccgg

SEQ ID NO: 221 - DNA, 22 bp, Artificial Sequence
  Description of Artificial Sequence: Synthetic oligonucleotide
  modified_base (14)..(14): dNaM
tcacacaatgtatngatcacgg

SEQ ID NO: 222 - DNA, 22 bp, Artificial Sequence
  Description of Artificial Sequence: Synthetic oligonucleotide
  modified_base (14)..(14): dTPT3
tcacacaatgtatnaatcacgg

SEQ ID NO: 223 - DNA, 22 bp, Artificial Sequence
  Description of Artificial Sequence: Synthetic oligonucleotide
  modified_base (12)..(12): dTPT3
accaggatgggnaccaccccgg

SEQ ID NO: 224 - DNA, 22 bp, Artificial Sequence
  Description of Artificial Sequence: Synthetic oligonucleotide
  modified_base (13)..(13): dNaM
attcacaatactntctttaagg

SEQ ID NO: 225 - protein, 22 aa, Artificial Sequence
  Description of Artificial Sequence: Synthetic peptide
MKYLLPTAEAGLLLLAAQPAIA

SEQ ID NO: 226 - protein, 26 aa, Artificial Sequence
  Description of Artificial Sequence: Synthetic peptide
MKIKTGARILALSELTTMMFSASALA

SEQ ID NO: 227 - protein, 21 aa, Artificial Sequence
  Description of Artificial Sequence: Synthetic peptide
MKQSTIALALLPLLFTPVTKA

SEQ ID NO: 228 - protein, 30 aa, Artificial Sequence
  Description of Artificial Sequence: Synthetic polypeptide
MKSPAPSRPQKMALIPACIFLCFAALSVQA

SEQ ID NO: 229 - protein, 20 aa, Artificial Sequence
  Description of Artificial Sequence: Synthetic peptide
MKKILVSFVAIMAVASSAMA

SEQ ID NO: 230 - protein, 40 aa, Artificial Sequence
  Description of Artificial Sequence: Synthetic polypeptide
MKISMQKADFWKKAAISLLVFTMFFTLMMSETVFAAGLNK

SEQ ID NO: 231 - protein, 28 aa, Artificial Sequence
  Description of Artificial Sequence: Synthetic peptide
MKKTAIAIAVALAGFATVAQASAGLNKD

SEQ ID NO: 232 - protein, 19 aa, Artificial Sequence
  Description of Artificial Sequence: Synthetic peptide
MKKIWLALAGLVLAFSASA

SEQ ID NO: 233 - DNA, 57 bp, Artificial Sequence
  Description of Artificial Sequence: Synthetic oligonucleotide
atgaaaaagatttggctggcgctggctggtttagttttagcgtttagcgcatcggcg

SEQ ID NO: 234 - protein, 22 aa, Artificial Sequence
  Description of Artificial Sequence: Synthetic peptide
MKYLLPTAAAGLLLLAAQPAMA

SEQ ID NO: 235 - DNA, 66 bp, Artificial Sequence
  Description of Artificial Sequence: Synthetic oligonucleotide
atgaaatacctgctgccgaccgctgctgctggtctgctgctcctcgctgcccagccggcgatggcg

SEQ ID NO: 236 - DNA, 63 bp, Artificial Sequence
  Description of Artificial Sequence: Synthetic oligonucleotide
atgaaacaaagcactattgcactggcactcttaccgttactgtttacccctgtgacaaaagcg

SEQ ID NO: 237 - protein, 26 aa, Artificial Sequence
  Description of Artificial Sequence: Synthetic peptide
MKTHIVSSVTTTLLLGSILMNPVANA

SEQ ID NO: 238 - DNA, 78 bp, Artificial Sequence
  Description of Artificial Sequence: Synthetic oligonucleotide
atgaaaacacatatagtcagctcagtaacaacaacactattgctaggttccatattaatgaatcctgtcgctaatgcc

SEQ ID NO: 239 - protein, 21 aa, Artificial Sequence
  Description of Artificial Sequence: Synthetic peptide
MKYLLPWLALAGLVLAFSASA

SEQ ID NO: 240 - DNA, 63 bp, Artificial Sequence
  Description of Artificial Sequence: Synthetic oligonucleotide
atgaaatacctgctgccgtggctggcgctggctggtttagttttagcgtttagcgcatcggcg

SEQ ID NO: 241 - protein, 20 aa, Artificial Sequence
  Description of Artificial Sequence: Synthetic peptide
MKKITAAAGLLLLAAFSASA

SEQ ID NO: 242 - DNA, 60 bp, Artificial Sequence
  Description of Artificial Sequence: Synthetic oligonucleotide
atgaaaaagattaccgctgctgctggtctgctgctcctcgctgcgtttagcgcatcggcg

SEQ ID NO: 243 - protein, 19 aa, Artificial Sequence
  Description of Artificial Sequence: Synthetic peptide
MKKIWLALAGLVLAQPAMA

SEQ ID NO: 244 - DNA, 57 bp, Artificial Sequence
  Description of Artificial Sequence: Synthetic oligonucleotide
atgaaaaagatttggctggcgctggctggtttagttttagcccagccggcgatggcg

SEQ ID NO: 245 - protein, 19 aa, Artificial Sequence
  Description of Artificial Sequence: Synthetic peptide
MKKILVLGALALWAQPAMA

SEQ ID NO: 246 - DNA, 57 bp, Artificial Sequence
  Description of Artificial Sequence: Synthetic oligonucleotide
atgaaaaagattttagttttaggtgctctggcgctgtgggcccagccggcgatggcg

SEQ ID NO: 247 - protein, 19 aa, Artificial Sequence
  Description of Artificial Sequence: Synthetic peptide
MKKIWLALVLLAGAQPAMA

SEQ ID NO: 248 - DNA, 57 bp, Artificial Sequence
  Description of Artificial Sequence: Synthetic oligonucleotide
atgaaaaagatttggctggcgttagttttactggctggtgcccagccggcgatggcg

SEQ ID NO: 249 - protein, 19 aa, Artificial Sequence
  Description of Artificial Sequence: Synthetic peptide
MKKILAGWLALVLAQPAMA

SEQ ID NO: 250 - DNA, 57 bp, Artificial Sequence
  Description of Artificial Sequence: Synthetic oligonucleotide
atgaaaaagattctggctggttggctggcgttagttttagcccagccggcgatggcg

SEQ ID NO: 251 - protein, 19 aa, Artificial Sequence
  Description of Artificial Sequence: Synthetic peptide
MKKILVLLAGWLAAQPAMA

SEQ ID NO: 252 - DNA, 57 bp, Artificial Sequence
  Description of Artificial Sequence: Synthetic oligonucleotide
atgaaaaagattttagttttactggctggttggctggcggcccagccggcgatggcg

SEQ ID NO: 253 - protein, 20 aa, Artificial Sequence
  Description of Artificial Sequence: Synthetic peptide
MKKITAAAGLLLLAAQPAMA

SEQ ID NO: 254 - DNA, 60 bp, Artificial Sequence
  Description of Artificial Sequence: Synthetic oligonucleotide
atgaaaaagattaccgctgctgctggtctgctgctcctcgctgcccagccggcgatggcg

SEQ ID NO: 255 - protein, 20 aa, Artificial Sequence
  Description of Artificial Sequence: Synthetic peptide
MKKILLLLGTAAAAAQPAMA

SEQ ID NO: 256 - DNA, 60 bp, Artificial Sequence
  Description of Artificial Sequence: Synthetic oligonucleotide
atgaaaaagattctgctgctcctcggtaccgctgctgctgctgcccagccggcgatggcg

SEQ ID NO: 257 - protein, 20 aa, Artificial Sequence
  Description of Artificial Sequence: Synthetic peptide
MKKILLLLLLLLLLAQPAMA

SEQ ID NO: 258 - DNA, 60 bp, Artificial Sequence
  Description of Artificial Sequence: Synthetic oligonucleotide
atgaaaaagattctgctgctcctcctgctgctcctcctgctcgcccagccggcgatggcg

SEQ ID NO: 259 - protein, 20 aa, Artificial Sequence
  Description of Artificial Sequence: Synthetic peptide
MKKIAAAAAAAAAAAQPAMA

SEQ ID NO: 260 - DNA, 60 bp, Artificial Sequence
  Description of Artificial Sequence: Synthetic oligonucleotide
atgaaaaagattgctgctgctgctgcggcggcggcggctgcggcccagccggcgatggcg

SEQ ID NO: 261 - protein, 21 aa, Artificial Sequence
  Description of Artificial Sequence: Synthetic peptide
MKYLLPWLALAGLVLAQPAMA

SEQ ID NO: 262 - DNA, 63 bp, Artificial Sequence
  Description of Artificial Sequence: Synthetic oligonucleotide
atgaaatacctgctgccgtggctggcgctggctggtttagttttagcccagccggcgatggcg

SEQ ID NO: 263 - protein, 22 aa, Artificial Sequence
  Description of Artificial Sequence: Synthetic peptide
MKYLLPTAAAGLLLLAAFSASA

SEQ ID NO: 264 - DNA, 66 bp, Artificial Sequence
  Description of Artificial Sequence: Synthetic oligonucleotide
atgaaatacctgctgccgaccgctgctgctggtctgctgctcctcgctgcgtttagcgcatcggcg